European Patent Application EP 4 610 366 A1, published September 3, 2025. Title: LENTIVIRUS INTEGRATION JUNCTION ANALYSIS. Applicant: Miltenyi Biotec BV Co KG. Application EP, filed February 29, 2024. The sequence listing filed with the application follows.

SEQUENCE LISTING (8 sequences)

SEQ ID NO: 1 - DNA, 94 bp, unidentified
  source 1..94: mol_type = genomic DNA
acacgacgctcttccgatcttgtcttcgttgggagtgaattagcccttccacagtacaagcaaaaagcagatctagatcggaagagcacacgtc

SEQ ID NO: 2 - DNA, 94 bp, unidentified
  source 1..94: mol_type = genomic DNA
tgtgctgcgagaaggctagaacagaagcaaccctcacttaatcgggaaggtgtcatgttcgtttttcgtctagatctagccttctcgtgtgcag

SEQ ID NO: 3 - DNA, 43 bp, unidentified
  source 1..43: mol_type = genomic DNA
acacgacgctcttccgatcttgtcttcgttgggagtgaattag

SEQ ID NO: 4 - DNA, 43 bp, unidentified
  source 1..43: mol_type = genomic DNA
gacgtgtgctcttccgatctagatctgctttttgcttgtactg

SEQ ID NO: 5 - DNA, 94 bp, unidentified
  source 1..94: mol_type = genomic DNA
acacgacgctcttccgatctcccttttagtcagtgtggaaaatctctagcactggtaactagagatccctcagaagatcggaagagcacacgtc

SEQ ID NO: 6 - DNA, 94 bp, unidentified
  source 1..94: mol_type = genomic DNA
tgtgctgcgagaaggctagagggaaaatcagtcacaccttttagagatcgtgaccattgatctctagggagtcttctagccttctcgtgtgcag

SEQ ID NO: 7 - DNA, 43 bp, unidentified
  source 1..43: mol_type = genomic DNA
acacgacgctcttccgatctcccttttagtcagtgtggaaaat

SEQ ID NO: 8 - DNA, 43 bp, unidentified
  source 1..43: mol_type = genomic DNA
gacgtgtgctcttccgatcttctgagggatctctagttaccag